European Patent Application EP 4 477 079 A1, published December 18, 2024. Title: METHOD FOR GENERATING A HUMANIZED ANIMAL MODEL OF A MENTAL DISORDER FROM THE HUMAN OLFACTORY NEUROEPITHELIUM. Applicant: UNIVERSIDAD DE CÁDIZ. The sequence listing filed with the application follows.

SEQUENCE LISTING (6 sequences)

SEQ ID NO: 1 - DNA, 24 bp, synthetic construct
  source 1..24: mol_type = other DNA
gggaagagagaggtgatggaacca

SEQ ID NO: 2 - DNA, 22 bp, synthetic construct
  source 1..22: mol_type = other DNA
aagccctgaaccctctctttgc

SEQ ID NO: 3 - DNA, 25 bp, synthetic construct
  source 1..25: mol_type = other DNA
ttggtggtgccgagtgagaagaaga

SEQ ID NO: 4 - DNA, 25 bp, synthetic construct
  source 1..25: mol_type = other DNA
gtctgggcagtggttggttggttaa

SEQ ID NO: 5 - DNA, 19 bp, synthetic construct
  source 1..19: mol_type = other DNA
cagattggctacccaactg

SEQ ID NO: 6 - DNA, 19 bp, synthetic construct
  source 1..19: mol_type = other DNA
gggaaggtgtaatccgtct